European Patent Specification EP 3 684 784 B1, published March 27, 2024. Title: NOVEL PEPTIDE AS POTENT INHIBITOR OF PROTEIN AGGREGATION. Applicant: Council of Scientific and Industrial Research Sharma, Deepak Kumar Gupta, Arpit Raghava, Gajendra Pal Singh Gautam, Ankur Kumari, Manisha. The sequence listing filed with the application follows.

SEQUENCE LISTING (3 sequences)

SEQ ID NO: 1 - protein, 4 aa, Artificial Sequence
  Sequence retrieved through Sequence logo
HHHH

SEQ ID NO: 2 - protein, 13 aa, Artificial Sequence
  Sequence retrieved through phage display screen; N terminal acetylation; Cys at 3rd position and 11th position can either be cysteine or cystine
SACNHHHHLHCGG

SEQ ID NO: 3 - protein, 13 aa, Artificial Sequence
  Sequence retrieved through phage display screen;N terminal acetylation;Cys at 3rd position and 11th position can either be cysteine or cystine
SACQHHHHHSCGG